European Patent Application EP 4 492 061 A1, published January 15, 2025. Title: SEX-SPECIFIC SPERM MEMBRANE PROTEINS FOR SPERM SEXING. Applicant: Universidade de Trás-os-Montes e Alto Douro (UTAD). Application EP, filed February 29, 2024. The sequence listing filed with the application follows.

SEQUENCE LISTING (34 sequences)

SEQ ID NO: 1 - protein, 1002 aa, Rabbit
MFFSGGQCGHVGRMEDILAAFRIALAVMCLHVVLVTSLEENADNSSLLLPPEVQTTSLNDATSSVLSTLNKTEKTKITIVKTFNASGIKPQKNICNLSSICNDSAFFRGEITFQYDEESNNTQNQDRANGTLNGMLSLSELKRSELNKTLQALSETYFIVCATAEAQSTQNCTFTVKLNTTMNICAIMAALKGVKIRPMEQCCCSVRTPCPSSPEDLEKLQCDLQDPVVCLPDHPQGPPFSSSSKPFPVGPQATVVSQVSSAFSMAEPVDNLQVTQKAHSAPGRGHLAPSQPSAPVASHPSIGLPPLQSGTLSPPVPQTNLSHTPPPVKSSFASPTKAAPANATSALPDKTNIINITSVSDLENQVSQMEKALSLGSLETDYAGEMINQVSKLLRSPPALLAPLAQRLLKVVDDIGLQLNFSNKTISLTSPSLALAVVRVNASNFDTTTFAAQDPANLQVSLETQAPENSIGIITLPSSLMSTIPANDMQLASRIQFNFFETPALFQDPSLENLSLISYVISSSVANLTIRNLTRNVTVTLKHIDQSQDALTVRCVFWDLGKNGGRGGWSTNGCSVKGQRLNETICTCNHLTSFGVLLDLSRTSLPPAQMMALTFITYIGCGLSSIFLSVTLVTYIAFEKIRRDYPSKILIQLCAALLLLNLVFLLDSWVALYNTRGFCISVAGFLHYFLLVSFTWMGLEAFHMYLALVKVFNTYIRKYILKFCIIGWGLPAVVVTIVLTISPDNYGLGSYGKFPNGSPDDFCWINSNVVFYITVVGYFCVVFLLNLSMFIVVLVQLCRIKRKKQLGAQRKTSIQDLRSIAGLTFLLGITWGFAFFAWGPVNVAFMYLFAIFNTLQGFFIFLFYCVAKENVRKQWRRYLCCGKLRLAENSDWSKTATNGLKKQTVNQGVSSSSNSLQSNSNSTNSTTLLVNNDCSVHASGNGNASTEKNGVSFSVQNGDVCLHDFTGKQHTFNEKDDSCNGKSRMTLRRTSKRGSLPFVEQM

SEQ ID NO: 2 - protein, 350 aa, Rabbit
MAVLVVLLSVLVAGVLGNEFSILRSPGSVVFRNGNWPIPGERIPDVAALSMGFSVKEDLSWPGLAVGDLFHRPRATVMVVVKGVDKLALPPGSVISYPLENAVPFSLDSVANSIHSLFSEETPVVLQLAPSEERVYMVGKANSVFEDLSVTLRQLRNRLFQESSILNSLPLNSLSRNNEVDLLFLSELQVLQDISSLLSRHKHLAKDHSPDLYSLELAGLDEIGKRYGEESEQFQDASRILVDALQKFADDMYNLYGGNAVVELVTVKSYDPSLVRKTRTILETRQENPTTPYNLAYKYNFEYSVVFNMVLWIMIALALAVIVTSYNIWNMDPGYDSIIYRMTNQKIRMD

SEQ ID NO: 3 - protein, 406 aa, Rabbit
MVFAFWKVFLILNCLIGQVRVVQVIIPEGFVNVTVGSDATLVCLYKTTVTSQDKLTIQWSFFHKKELEPISHSPCLNTEGMEEKAVSQCLKMAHARDARGRCSWTSQIYYSEGGQAAAIGRFKDRIIGTNNPSNASITILNMQPADSGIYICDVNNPPDFAGRNQGIVNVSVLVKPSKPFCSIQGRPEAGHAISLSCLSALGTPSPVYYWYKLEGTNIVPVKESFNPATGILDIGNLTNFEQGYYQCTAINMLGNSSCEIDLTSSHPEVGIIIGALIGTLVGAAIIASVVCFARNKSKAKDRKRNTKATTELEPMTQKTQRAGTEAMPTEDVVQLEAALPPSTHETDPATIMEPDHELPRPEGVQRQGPVLQPELEIELEPEPVLEPEPGIAAESQRDEKKRVVKP

SEQ ID NO: 4 - protein, 246 aa, Rabbit
MSLQWTAVATFLYAEVFAVLLLCIPFISPKRWQKIFKSRLVELVVTYGNTFFVVLISILVLLVIDAVREIRKYDDVTEKVNLQNNPGAMEHFHMKLFRAQRNLYIAGFSLLLSFLLRRLVTLISQQATLLASNEAFKKQAESASEAAKKYMEENDQLKKGAAVDRRKLDVGDTEVKLEEENRSLKANLKKLKDDLASAKQKLEKAENEALAMRKQSEGLTKEYDRLLDEHAKLQASVDGTTDKKEE

SEQ ID NO: 5 - protein, 195 aa, Rabbit
MAAEDVVATGADLSELEGGGLLHEIFTSPLNLLLLGLCIFLLYKIVRGDQPGASSDSDDEEPPPLPRLKRRDFTPAELRRFDGVQDPRILMAINGKVFDVTKGRKFYGPEGPYGVFAGRDASRGLATFCLDKEALKDEYDDLSDLTPAQRETLSDWDSQFTFKYHLVGKLLKEGEEPTVYSDEDEPKDETARKND

SEQ ID NO: 6 - protein, 348 aa, Rabbit
MSSSSPQLPEMEPSSSGPSSYKVGTMAEKFDCHYCRDPLQGKKYVQKDGHHCCLKCFDKFCANTCAECRKPIGADSKEVHYKNRYWHDTCFRCAKCLRSLASETFVAKDNKIYCNKCATREDSPKCKGCFKAIVAGDQNVEYKGTIWHKDCFTCSNCKQVIGTGSFFPKGEDFYCVTCHETKFAKHCVKCNKAITSGGITYQDQPWHADCFVCVTCSKKLAGQRFTAVEDQYYCVDCYKNFVAKKCAGCKNPITGKRTVSRVSHPVSKARKPPVCHGKRLPLTLFPSANLRGRHPGGERTCPSWVVVLYRKNRSLAAPRGPGLVKAPVWWPMKDNPGTTTASTAKNAP

SEQ ID NO: 7 - protein, 630 aa, Rabbit
MDEMATTQISKDELDELKEAFAKVDLNSNGFICDYELHELFKEANMPLPGYKVREIIQKLMLDGDRNKDGKISFDEFVYIFQEVKSSDIAKTFRKAINRKEGICALGGTSELSSEGTQHSYSEEEKYAFVNWINKALENDPDCRHVIPMNPNTDDLFKAVGDGIVLCKMINLSVPDTIDERAINKKKLTPFIIQENLNLALNSASAIGCHVVNIGAEDLRAGKPHLVLGLLWQIIKIGLFADIELSRNEALAALLRDGETLEELMKLSPEELLLRWANFHLENSGWQKINNFSADIKDSKAYFHLLNQIAPKGQKEGEPRIDINMSGFNETDDLKRAESMLQQADKLGCRQFVTPADVVSGNPKLNLAFVANLFNKYPALTKPENQDIDWTLLEGETREERTFRNWMNSLGVNPHVNHLYADLQDALVILQLYERIKVPVDWSKVNKPPYPKLGANMKKLENCNYAVELGKHPAKFSLVGIGGQDLNDGNQTLTLALIWQLMRRYTLNVLEDLGEGQKANDDIIVNWVNRTLSEAGKSTSIQSFKDKTISSSLAVVDLIDAIQPGCINYDLVKSGNLTEDDKHNNAKYAVSMARRIGARVYALPEDLVEVKPKMVMTVFACLMGRGMKRV

SEQ ID NO: 8 - protein, 662 aa, Rabbit
MSHVAVENALGLDQQFAGLDLNSSDNQTGGSTASKGRYIPPHLRNREATKGFYDKDSSGWSSSKDKDAYSSFGSRGDSRGKSSFFSDRGSGSRGRFDDRGRGDYDGIGSRGDRSGFGKFERGGNSRWCDKSDEDDWSKPLPPSERLEQELFSGGNTGINFEKYDDIPVEATGNNCPPHIESFSDVEMGEIIMGNIELTRYTRPTPVQKHAIPIIKEKRDLMACAQTGSGKTAAFLLPILSQIYSDGPGEALRAMKENGRYGRRKQYPISLVLAPTRELAVQIYEEARKFSYRSRVRPCVVYGGADIGQQIRDLERGCHLLVATPGRLVDMMERGKIGLDFCKYLVLDEADRMLDMGFEPQIRRIVEQDTMPPKGVRHTMMFSATFPKEIQMLARDFLDEYIFLAVGRVGSTSENITQKVVWVEESDKRSFLLDLLNATGKDSLTLVFVETKKGADSLEDFLYHEGYACTSIHGDRSQRDREEALHQFRSGKSPILVATAVAARGLDISNVKHVINFDLPSDIEEYVHRIGRTGRVGNLGLATSFFNERNVNITKDLLDLLVEAKQEVPSWLENMAYEHHYKGSSRGRSKSSRFSGGFGARDYRQSSGASSSSFSSSRASSSRSGGGGHGGSRGFGGGGYGGFYNSDGYGGNYNSQGVDWWGN

SEQ ID NO: 9 - protein, 745 aa, Bovine
MLCLLFLLLGLTGLQTDDNSERLRVQFTVPEKIRSTSSGGVETHVSYIILIEGKTYTVNLMQKAFLPHNFRVYGYSGTGSMKPLEHEFQNFCYYQGYIEGYPNSMAIISTCTGLRGLLQFENVSYGIEPLEPSIGFEHMVYQIKPRDSSSSVYTEREIELREKPYKIQNVEPLPDFSQYIEMHIVVEKDLYNHMGADTTVVIQKIFQLTGLTNAIFTSLNITVILSSLELWIDENKIPVTGDANELLHRFVKWKRSYLVLRPHDMAFLLVYREKSNYIGATFQGRMCDKHYGGGVALHSSTISLESLAVIIAQLLSLSMGIPYDDINKCHCPGDVCIMNPAAVHSSGVKLFSNCSVEDFLRFISKPKSQCLQNQPRLDPTYKSAVCGNGKVEEGEQCDCGNKKACDALPDTCCVADTCRFQPGSACDTGLCCESCAFIPKGHICRGSTDECDLHEYCNGSSAACQEDVYVQDGHPCGQNQWLCISGICVDGIKQCFDIFGEGTSYAPAECFQRLNSMNDLSGNCGVTPTGFTPCTSENVRCGKLLCTYDKREVISVENASVMYSNINGKICIGLHYEYGNEDEGMMWVKDGTVCGESKICQNKQCVDSSFLNYDCNPEKCNNQGVCNNKKHCHCNPSYLPPNCEHSAPGWEGGSIDSGNFPPSEPPTGGPAFTDVGTTPLAESRYIENVYRSKPTRWPFFLFIPFFIILCVLIATLVKVYFQRKKWRTEDYTSDEQLESESEPKD

SEQ ID NO: 10 - protein, 1119 aa, Bovine
MQRVPPSSPASECAGEEKRVGTRTVFVGNHPVSETEAYIAQKFCDNRIISSKYTLWNFLPKNLFEQFRRIANFYFLIIFLIQVTVDTPTSPITSGLPLFFVITVTAIKQGYEDWLRHRADNEVNKSTVYIIENAKRVKKESEKIKVGDIVEVQADETFPCDLILLSSCTVDGTCYVTTASLDGESNCKTHYAVRDTIELRTVESIDNLRAAIECEQPQPDLYKFVGRINIYSNSIEAVARSLGPENLLLKGATLKNTKKIYGVAVYTGMETKMALNYQGKSQKRSAVEKSINAFLIVYLFILLTKAAICTTLKYVWQSTPHNDEPWYNQKTQKERETWKVLKMFTDFLSFMVLFNFIIPVSMYVTVEMQKFLGSFFISWDNDFYDEEINEGALVNTSDLNEELGQVDYVFTDKTGTLTENTMEFIECCIDGHKYKGVAQETDGLSQTDGPLPYLDRADKNREELFLRALCLCHTVEVKPNDTVDGVTESSELTYMSSSPDEIALVKGAKKYGFTFVGVQNGYMRVENQRKEIEEYELLHTLNFDAVRRRMSVIVKTQTGDILLFCKGADSAVFPRVQNHEIDLIKVHVEHNAMEGYRTLCIAFKEIAPDDYERVNRQLIEAKMALQDREEKMEKVFDEIETDMHLIGATAVEDKLQDQAAETIEALHAAGLKVWVLTGDKMETAKSTCYACRLFQTNTELLELTTKTIEESERKEDRLHELLTEYRKKLLHEFPKSTRSLKKAWTEHQEYGLIIDGSTLSLILNSSQDSGSNNYKSIFLQICMKCTAVLCCRMAPLQKAQIVRMVKNLKGSPITLSIGDGANDVSMILESHVGIGIKGKEGRQASRNSDYAVPKFKHLKKLLLAHGHLYYVRIAHLVQYFFYKNLCFILPQFLYQFFCGFSQQPLYDAAYLTMYNICFTSLPILAYSLLEQHINIDTLTSDPRLYMKISGNAMLQLGPFLYWTFLAAFEGTVFFFGTYFLFQTTSLDENGKVYGNWTFGTIIFTILVFTVTLKLALDTRFWTWINHLVIWGSLAFYVFFSFFWGGIIWPFLKQQRMYFVFAQMLSSVSVWLTIILLIFVSLSPEMLRIVLRSVRRRSTRNPNLELPMLLSYKHIDSGYR

SEQ ID NO: 11 - protein, 1043 aa, Bovine
MNWPFFRAAVVLFIFLVVLEVNSDFRIQVRDYNTKNGTIKWHSLRRQKREWIKFAAACREGEDNSKRNPIAKIHSDCAANQQVTYRISGVGIDQPPYGIFVINQKTGEINITSIVDREVTPFFIIYCRALNSLGQDLEKPLELRVRVLDINDNPPVFSMSTFVGEIEENSNANTLVMVLNATDADEPNNLNSKIAFKIIRQEPSDSPMFIINRYTGEIRTMNNFLDREQYGQYSLAVRGSDRDGGADGMSAECECNIKILDVNDNIPYMELPTQSISIEENSLNSNLLQIRVIDLDEEFSANWMAVIFFISGNEGNWFEIEMNERTNVGTLKVVKPLDFEAMNNLQLSLGVRNKAEFHQSIMSQYKLTATAISVTVLNVVEGSVFRPGSKTFVVNSNMGQNYKIGEYVAWDLDANRPSTTVRYVMGRNPTDLLAIDSKTAIITLRNKVTMEQYKILGGKYQGTILSIDDALQRTCTGTIVINLENGGWKTERPNVNGSTTSAYGLTSGGVTTNGYTTGGGVGTVTFAVGTNGYGVGTGVYQPLRDNVHFGPAGIGLLIMGFLVLGLVPFLLMCCDCGGAPGGGAAFEPVPECSDGAIHSWAVEGAQADPGVLANSAVPCIPVTNANVIEYVDNSGVYTNEYGAREMQDLGGGERTTGFELTDGVKMSGGPEICQEYPGTLRRNSMRECREGGLNMNFMESYFCQKAYAYADEDEGRPSNDCLLIYDIEGAGSPAGSVGCCSFIGEDLDDSFLDTLGPKFKKLADISLGKDVEPFPDSDPSWPPKSTEPVCPPQGTEPTGGGHPPISPRFGTTTVISENTYPSGPGVQHPTPIPDPLGYGNVTVTESYTSSGTLKPSVHIHDNRHASNVVVTERVVGPISGADLQGMLEMPDLRDGSNVIVTERVIAPSSSLPTTLTIPDPRQSSNVVVTERVIQPTSGIVGNLSMHPELSNTHNVIVTERVVSGSGITGSSSLLGSAGGGSGGGIGLGSLGGGGGLSSSLGGAATIGHLRGSAEHHFSNTLGSASPTTTRSRITKYSTVQYTK

SEQ ID NO: 12 - protein, 1043 aa, Bovine; identical to SEQ ID NO: 11

SEQ ID NO: 13 - protein, 1207 aa, Bovine
MTNPTEHTLPSNSILESREGEFGCTVMDLRKLMELRSSDAIDQINVHYGGVMNLCSRLKTNPVEGLSGNPADLEKRKQVFGQNLIPPKKPKTFLELVWEALQDVTLIILEIAAIISLVLSFYRPPGGENEQCGLAVTSPEDEGEAEAGWIEGAAILFSVIIVVLVTAFNDWSKEKQFRGLQNRIEKEQKFSVIRNGHIIQLPVAEIVVGDIAQIKYGDLLPADGILIQGNDLKIDESSLTGESDHVKKSLERDPMLLSGTHVMEGSGRMVVTAVGINSQTGIIFTLLGASEGEEEEKKKKGKKQGVPENRNKAKTQDGVALEIQPLNSQEGIDSEEKEKKAAKLPKKEKSVLQGKLTRLAVQIGKAGLIMSAITVLILILYFVIDNFVIQRRPWLAECTPIYVQYFVKFFIIGVTVLVVAVPEGLPLAVTISLAYSVKKMMKDNNLVRHLDACETMGNATAICSDKTGTLTMNRMSVVQAYIGDTRYHQIPSPDDLVPKVLDLIVNGISINSAYTSKILPPEKEGGLPRQVGNKTECALLGFVSDLKQDYHAVRSEVPEEKLYKVYTFNSVRKSMSTVIEKPGGGYRMYSKGASEIILRKCNRILDKKGEAVPFKNKDRDEMVRTVIEPMACEGLRTLCIAYRDFNDGEPPWDNESEILTELTCIAVVGIEDPVRPEVPEAIAKCKRAGITVRMVTGDNINTARAIATKCGIVTPGDDFLCLEGKEFNRLIRNEKGEVEQEKLDKIWPKLRVLARSSPTDKHTLVKGIIDSTVGDQRQVVAVTGDGTNDGPALKKADVGFAMGIAGTDVAKEASDIILTDDNFTSIVKAVMWGRNVYDSISKFLQFQLTVNVVAVIVAFTGACITQDSPLKAVQMLWVNLIMDTFASLALATEPPTDSLLKRRPYGRNKPLISRTMMKNILGHAVYQLTVIFFLVFAGEKFFDIDSGRRAPLHSPPSQHYTIIFNTFVLMQLFNEINSRKIHGERNVFSGIFRNLIFCSVVLGTFISQIIIVEFGGKPFSCTKLTLSQWFWCLFIGIGELLWGQVISTIPTQSLKFLKEAGHGTTKEEITKDAEGLDEIDHAEMELRRGQILWFRGLNRIQTQIKVVKAFHSSLHESIQKPKNQNSIHNFMTHPEFTIDEEGPRTPLLDEQEEEIFEKVSKPGTKTSSLDGEVTPQTNKNNNTVDCCQVQIVASHSDSPLHSLETSV

SEQ ID NO: 14 - protein, 848 aa, Bovine
MSDDIDWLHSRRGVCKVDLYSPRGQQDQDRKVICFVDVSTLSMEDKDSKDAAGCSSEGDLNLENLEEKEIIVIKDTEKQDQSKTEGSVCLFKQAPSDPLSVFNWLLNDLQKYALGFQHALSPSASSCKHKVGETEGNCQKLSSGNCYSIYANHLNMDCVNNEPQSLRLEMTAAKNTNNNQSPSTPPGKSPSNQRAVISPDGECSMDDLSFYVNRLSSLVIQMARKEIKEKLENGSKCLHHSIYPPSGDKGKNSPRSAVSKIASEMAHDAVEVTSAEMRGTGEECRDGGRKTFLYSELSNKNKGGDKQMCQRDSKDFADSISKGLMVYANQVASDMMVSVMKTLKVHSSGKPIPACVVLKRVLLKHTKEIVSDLIDSCMKNLHNITGVLMTDSDFVSAVKRNLFNHGKQNAADIMEAMLKRLVSALLGEKKETKSQCLSYTSLKAGSHDAKCKNQSLEFSSVKAEMKGKDKCKVKQEECKSLTSAEKVSEHILKESLTMWNQKQCNQGKMPSKTCPHKEEKREKISPSTDSLAKDLIVSALMLIQYHLTQQAKGKEACEDDCPPGTTSYMTQSAQYEKCGGSQSAKALSMKHLETRGAPGPSTSMKDNQHLDSQKLDMSNMVLSLIQKLLNESPFNCEDLCEGENKHSEIRTNKSTSIFKKSDREEEQGQDNREVDFVGGMKQVNRQFIDQLVESVMKLCLIMAKYSNNEAALTDLEEQASSSNNSNFYQTSGPRSSYEAGMSQSYQDSHGPEVIVNNQCSTSSLQKQLQAVLQWIAASQFNVPMLYFMGDDDGQLEKLPEVSAKAAEKGYSVGDLLQEVMKFAKERQLDEAVGNMARKQLLDWLLANL

SEQ ID NO: 15 - protein, 667 aa, Bovine
MSLPRLCLGELINEDIHTWNSLCRQEITIKTYDNSIPISESSKKIRNQQYLTITFPKSSQPGGNKRLRPSEIQVTVPRHDKRNLDELQKPAHIWIRHSLRKKFQSPSINLIVRRQASFRHPYTHITHSKKAESKKYKDDKKETALKKISKKDTGPHEVDEKPKRRNKADKTPSKSSHGSQLSKKSKSKSETNPESKDSISVSIKHQKKEKRYSKDSKEMDFESTSTKKYSKSSKNNSDAVSETCSKNSSNVGLMVHLGESDAESMEFDMWLKNYSQNNSKKPTKKDAKKDAKGKGSDAESVDSKDAKKDKKGATKDTKKGAKKDTESTDAESGDSKDAKKGKKESKKDKKKDAKKDAASDAESGDSKDAKKDSKKGKKDSKKDNKKKDAKKDAESTDAESGDSKDAKKDSKKGKKDSKKDDKKKDAKKDAESTDAESGDSKNAKKDSKKGKKDDKKKDAKKDAVSTDADSESEGDAKKSKKDSKKDKKDLKKDDQKKPAMKSKESTETESDWESKKVKRDSKKDTKKTAKKATESSGAESDVSSKRYLKKTEMFKSSDAESEESLFKPGSKKRVDESDATSTDSKKDAVEPKRGIKMPSRRTTFKEKGKKIGTGRVPPSRERPPLPPCEPILPSPRVKRLCRCQMPPPPPKPRYAPLPEAKWIHKLL

SEQ ID NO: 16 - protein, 190 aa, Bovine
METSTQRTGSHLAQTAAARHSASSRGEAARVSSRDELAEMAAASQGNFEGKFESLDLAELAKKQPWWRTLFGQESGPSAEKYSVATQLLIGGVTGWCTGFIFQKVGKLAATAVGGGFFLLQLANHTGYIKVDWQRVEKDMKKAKEQLKIRKSNQIPTEVKSKAEEVVSFVKKNVLVTGGFFGGFLLGMAS

SEQ ID NO: 17 - protein, 658 aa, Bovine alphaherpesvirus 1
MNTPNLEDMGCGTSSATKDKKSEKALKAALVIQNWYRGYSARLKTRQRYALTIFQSIEYADEQGQLQLSNFFSFMLENYTNVPEKEPGLVTRLFGSSIQDKDRQDYLGLIEIPDSYCGPRLQFPLTFTDIDLLIEAFKQQQILHAYYVLEVLFETKKVLQQMPNFTHTNTSPSKEITICGDLHGKLDDLFLIFYKNGLPSVTNPYVFNGDFVDRGKNSMEILMILFVSFLVYPNDLHLNRGNHEDFMMNMRYGFTKEILHKYKLHGKKILQILEEVYTWLPIGTIIDNEVLVIHGGISESTDLNLLHRIERNKMRSVLMPPIPMDGDRAEKKNKLGTATVALGIRTSGSFSEQLTKQEWEQVIDILWSDPRGKRGCYPNTNRGGGCYFGPDITSKILNKYQLKMLVRSHECKPEGYEICHDGKVITVFSASNYYEEGSNRGAYIRMSSGTTPRFFQYQITKATCFRPLYQRVNAIESSAIRMLKERMISRKTDLIRAFQLQDRNKSGKLSMGQWAFSMENVLGLNLPWRSLSSHLVTTDKDGNIDYMSGFQDVHIQKPVKEVQSSLIETVYRYRSDLQIIFNIIDSDHSGLISMEEFRSMWRLFKSHYSVHIDDSQFDELAERMDLNKDGSIDFNEFLKAFYVVHKFDQLNKSDTKLA

SEQ ID NO: 18 - protein, 434 aa, Bovine
MSILKVHAREIFDSRGNPTVEVDLFTAKGLFRAAVPSGASTGIYEALELRDNDKTRYMGKGVSKAVEHINKTIAPALVSKKLNVVEQEKIDKLMIEMDGTENKSKFGANAILGVSLAVCKAGAVEKGVPLYRHIADLAGNAEVILPVPAFNVINGGSHAGNKLAMQEFMILPVGAENFREAMRIGAEVYHNLKNVIKEKYGKDATNVGDEGGFAPNILENKEALELLKNAIGKAGYSDKVVIGMDVAASEFYRSGKYDLDFKSPDDPSRYITPDELANLYKSFIRDYPVVSIEDPFDQDDWEAWQKFTASAGIQVVGDDLTVTNPKRIAKAVSEKSCNCLLLKVNQIGSVTESLQACKLAQSNGWGVMVSHRSGETEDTFIADLVVGLCTGQIKTVAPCRSERLAKYNQILRIEEELGSKAKFAGRSFRNPLAK

SEQ ID NO: 19 - protein, 241 aa, Bovine
MILRKKLSYLWTLGLCLVASKSPPKAPSITNDRFIEECLRLHNEARTNVSPPAADMKYMSWDEALAKTAEAWAKKCKFIHNSCSSKSFKCHPTFQYAGENLWLGPLTISAAKFAINMWYDERKFYDFNTRSCSQVCGHYTQVVWAYSYKVGCAVAVCPNLGSPDSALLVCNYAPAGNYPNMSPYTNGTPCSMCQGDTCENNLCRNKERDKSQRYPNWNPSGTRQLIACNPLYLISVLLTIF

SEQ ID NO: 20 - protein, 641 aa, Bovine
MAAAKGTAIGIDLGTTYSCVGVFQHGKVEIIANDQGNRTTPSYVAFTDTERLIGDAAKNQVAMNPQNTVFDAKRLIGRKFNDPVVQSDMKLWPFQVINEGGKPKVMVSYKGEKKAFYPEEISSMVLTKMKETAEAFLGYTVTNAVITVPAYFNDSQRQATKDAGVIAGLNVLRIINEPTAAAIAYGLDKAGQGERHVLIFDLGGGTFDVSVLTIDDGIFEVKATAGDTHLGGEDFDNRLVSHFVEEFKRKHKKDISQNKRAVRRLRTACERAKRTLSSSTQANLEIDSLYEGIDFYTSITRARFEELCADLFRGTLEPVEKALRDAKMDKAKIHDIVLVGGSTRIPKVQRLLQDYFNGRDLNKSINPDEAVAYGAAVQAAILMGDKSEKVQDLLLLDVAPLSLGLETAGGVMTVLIKRNSTIPTKQTQIFTTYSDNQPGVLIQVYEGERAMTRDNNLLGRFDLTGIPPAPRGVPQIEVTFDIDANGILNVTAMDKSTGKANKITITNDKGRLSKEEIERMVLDAEKYKAEDEVQREKIAAKNALESYAFNMKSAVSDEGLQGKISESDKKKILSKCNEVLLWLEANQLAEKDEFDHKRKELEQVCNPIITKLYQGGCTGPSCGTGYTPGRAATGPTIEEVD

SEQ ID NO: 21 - protein, 650 aa, Bovine
MSKGPAVGIDLGTTYSCVGVFQHGKVEIIANDQGNRTTPSYVAFTDTERLIGDAAKNQVAMNPTNTVFDAKRLIGRRFDDAVVQSDMKHWPFMVVNDAGRPKVQVEYKGETKSFYPEEVSSMVLTKMKEIAEAYLGKTVTNAVVTVPAYFNDSQRQATKDAGTIAGLNVLRIINEPTAAAIAYGLDKKVGAERNVLIFDLGGGTFDVSILTIEDGIFEVKSTAGDTHLGGEDFDNRMVNHFIAEFKRKHKKDISENKRAVRRLRTACERAKRTLSSSTQASIEIDSLYEGIDFYTSITRARFEELNADLFRGTLDPVEKALRDAKLDKSQIHDIVLVGGSTRIPKIQKLLQDFFNGKELNKSINPDEAVAYGAAVQAAILSGDKSENVQDLLLLDVTPLSLGIETAGGVMTVLIKRNTTIPTKQTQTFTTYSDNQPGVLIQVYEGERAMTKDNNLLGKFELTGIPPAPRGVPQIEVTFDIDANGILNVSAVDKSTGKENKITITNDKGRLSKEDIERMVQEAEKYKAEDEKQRDKVSSKNSLESYAFNMKATVEDEKLQGKINDEDKQKILDKCNEIINWLDKNQTAEKEEFEHQQKELEKVCNPIITKLYQSAGGMPGGMPGGMPGGFPGGGAPPSGGASSGPTIEEVD

SEQ ID NO: 22 - protein, 338 aa, Bovine
MLSALARPAGAALRRSFSTSAQNNAKVAVLGASGGIGQPLSLLLKNSPLVSRLTLYDIAHTPGVAADLSHIETRATVKGYLGPEQLPDCLKGCDVVVIPAGVPRKPGMTRDDLFNTNATIVATLTAACAQHCPEAMICIISNPVNSTIPITAEVFKKHGVYNPNKIFGVTTLDIVRANAFVAELKDLDPARVNVPVIGGHAGKTIIPLISQCTPKVEFPQDQLTTLTGRIQEAGTEVVKAKAGAGSATLSMAYAGARFVFSLVDAMNGKEGVVECSFVKSQETDCPYFSTPLLLGKKGIEKNLGIGKVSPFEEKMIAEAIPELKASIKKGEEFVKNMK

SEQ ID NO: 23 - protein, 187 aa, Bovine
MPVDLSKWSGPLSLQEVDERPQHPLQVKYGGAEVDELGKVLTPTQVKNRPTSITWDGLDPGKLYTLVLTDPDAPSRKDPKYREWHHFLVVNMKGNNISSGTVLSDYVGSGPPKGTGLHRYVWLVYEQEGPLKCDEPILSNRSGDHRGKFKVASFRKKYELGAPVAGTCYQAEWDDYVPKLYEQLSGK

SEQ ID NO: 24 - protein, 279 aa, Bovine
MTKTDKKSFNQSLAEWKLFIYNRTTGEFLGRTAKSWGLILLFYLVFYGFLAALFSFTMWAMLQTLNDEVPKYRDQIPSPGLMVFPKPVSALDFSFSLSDAESYQGYIDDLKKFLKPYGLEEQKNLTDCTNGTFFEQKGPEYTACQFPLALLEACSGVDDPTFGYQEGKPCILVKMNRIIGLKPQGEPRIECTGKSESTAFLSTYPSNGTIDLKYFPYYGKKLHGNYLQPLVAVQVGFGSDADVREVMVECKIDGSPNLKTQNDRDKFLGRVAFKITMHA

SEQ ID NO: 25 - protein, 528 aa, Bovine
MLGLVGRVVAASASGALRGLSPSAPLPQAQLLLRAAPAALQPARDYAAQASPSPKAGATTGRIVAVIGAVVDVQFDEGLPPILNALEVQGRETRLVLEVAQHLGESTVRTIAMDGTEGLVRGQKVLDSGAPIRIPVGPETLGRIMNVIGEPIDERGPIKTKQFAAIHAEAPEFVEMSVEQEILVTGIKVVDLLAPYAKGGKIGLFGGAGVGKTVLIMELINNVAKAHGGYSVFAGVGERTREGNDLYHEMIESGVINLKDATSKVALVYGQMNEPPGARARVALTGLTVAEYFRDQEGQDVLLFIDNIFRFTQAGSEVSALLGRIPSAVGYQPTLATDMGTMQERITTTKKGSITSVQAIYVPADDLTDPAPATTFAHLDATTVLSRAIAELGIYPAVDPLDSTSRIMDPNIVGSEHYDVARGVQKILQDYKSLQDIIAILGMDELSEEDKLTVSRARKIQRFLSQPFQVAEVFTGHLGKLVPLKETIKGFQQILAGEYDHLPEQAFYMVGPIEEAVAKADKLAEEHS

SEQ ID NO: 26 - protein, 636 aa, Bovine alphaherpesvirus 1
MSARGPAIGIDLGTTYSCVGVFQHGKVEIIANDQGNRTTPSYVAFTDTERLIGDAAKNQVAMNPTNTIFDAKRLIGRKFEDATVQSDMKHWPFRVVSEGGKPKVQVEYKGEIKTFFPEEISSMVLTKMKEIAEAYLGGKVQSAVITVPAYFNDSQRQATKDAGTITGLNVLRIINEPTAAAIAYGLDKKGCAGGEKNVLIFDLGGGTFDVSILTIEDGIFEVKSTAGDTHLGGEDFDNSMVSHLAEEFKRKHKKDIAPNKRAVRRLRTACERAKRTLSSSTQASIEIDSLYEGVDFYTSITRARFEELNADLFRGTLEPVEKALRDAKLDKGQIQEIVLVGGSTRIPKIQKLLQDFFNGKELNKSINPDEAVAYGAAVQAAILIGDKSENVQDLLLLDVTPLSLGIETAGGVMTPLIKRNTTIPTKQTQTFTTYSDNQSSVLVQVYEGERAMTKDNNLLGKFDLTGIPPAPRGVPQIEVTFDIDANGILNVTAADKSTGKENKITITNDKGRLSKDDIDRMVQEAERYKSEDEANRDRVAAKNAVESYTYNIKQTVEDEKLRGKISDQDKNKILDKCQEVINWLDRNQMAEKDEYEHKQKELERVCNPIISKLYQGGPGGGGGSGASGGPTIEEVD

SEQ ID NO: 27 - protein, 655 aa, Bovine
MKLSLVAAVLLLLLGTARAEEEDKKEDVGTVVGIDLGTTYSCVGVFKNGRVEIIANDQGNRITPSYVAFTPEGERLIGDAAKNQLTSNPENTVFDAKRLIGRTWNDPSVQQDIKFLPFKVVEKKTKPYIQVDVGGGQTKTFAPEEISAMVLTKMKETAEAYLGKKVTHAVVTVPAYFNDAQRQATKDAGTIAGLNVMRIINEPTAAAIAYGLDKREGEKNILVFDLGGGTFDVSLLTIDNGVFEVVATNGDTHLGGEDFDQRVMEHFIKLYKKKTGKDVRKDNRAVQKLRREVEKAKRALSSQHQARIEIESFYEGEDFSETLTRAKFEELNMDLFRSTMKPVQKVLEDSDLKKSDIDEIVLVGGSTRIPKIQQLVKEFFNGKEPSRGINPDEAVAYGAAVQAGVLSGDQDTGDLVLLDVCPLTLGIETVGGVMTKLIPRNTVVPTKKSQIFSTASDNQPTVTIKVYEGERPLTKDNHLLGTFDLTGIPPAPRGVPQIEVTFEIDVNGILRVTAEDKGTGNKNKITITNDQNRLTPEEIERMVNDAEKFAEEDKKLKERIDTRNELESYAYSLKNQIGDKEKLGGKLSSEDKETMEKAVEEKIEWLESHQDADIEDFKAKKKELEEIVQPIISKLYGSAGPPPTSEEEAADKDEL

SEQ ID NO: 28 - protein, 573 aa, Bovine
MLRLPAVLRQMRPVSRALALHLTRAYAKDVKFGADARALMLQGVDLLADAVAVTMGPKGRTVIIEQSWGSPRVTKDGVTVAKSIDLKDKYKNIGAKLVQDVANNTNEEAGDGTTTATVLARSIAKEGFEKISKGANPVEIRRGVMLAVDAVIVELKKQSKPVTTPEEIAQVATISANGDKEIGNIISDAMKKVGRKGVITVKDGKTLNDELEIIEGMKFDRGYISPYFINTSKGQKCEFQDAYVLLSEKKISSVQSIVPALEIANAHRKPLVIIAEDVDGEALSTLVLNRLKVGLQVVAVKAPGFGDNRKNQLKDMAIATGGAVFGEEGLNLNLEDVQPHDLGKVGEVIVTKDDAMLLKGKGDKAQIEKRIQEIIEQLDITTSEYEKEKLNERLAKLSDGVAVLKVGGTSDVEVNEKKDRVTDALNATRAAVEEGIVLGGDCALLRCIPALESITPANEDQKTGIEIIKKTLKIPAMTIAKNAGVEGSLIVEKIMQSSSEVGYDAMLGDFVNMVEKGIIDPTKVVRTALLDAAGVASLLTTAEVVVTEIPKEEKDPGMGGMGGMGGGMGGGMF

SEQ ID NO: 29 - protein, 744 aa, Bovine
LLCPRWQTSLSSAPMPAEGWVSLRAALWLLGLCAVLAPVQCSPDRPSWRYISTEVVIPRKELHQGKGAQVLGWLSYSLRFRGQRHVIHMRRKRLFWPGYLMMTQDDQGVLQTDHPFVPEDCYYFGYLEEIPFSTVTINTCYGGLQGYMKLDDLAYEISPLKHSRKFEHTLSQMVADASTMGPMPRLGYEEERDPLLSPANITAAPRMSSKLYMFHEALMKGLCQSTNAFYRTANNVSETVQYMVDVGNIIDAVYRGLETRFYISVMHIYNVRDPVSTASLRRGSAYFQFYSRTLFPAFHPHTAVVFSTAEPPDGVYVPGLYSFCHSGGLVPIATSGKNTLTVALYVCFLIGRSIGLYYDYPDCVCQRRTTCIMNGYQSLTDAFSNCSYGHLQHIVMRDRSSCMFHPEPVYYNKSMTHERCGNKEVENEEQCDCGSFKECYSNPCCDNLCSFTEASICDADTCCTNCTFSKPGTLCRPIRSMCDLPEYCRGISKTCPRDVFMQDGTPCGEEGYCFKGTCTDRSVHCKEIFGRGALNAPDQCYTINRKAYRFGFCRRTSWSVRFIACSQQDQLCGRLQCTNVSFLPPLQEHVGFHQTHTLEALCFGLDLHRGQGAVDYGQVKNGALCAPGKYCLNTFCNGSVSKMEYTCFPQKCNSRGVCNSEDNCHCHLGWAPPFCENTGDGGSEDSGPPPRLFRSVPYDETILVYVRLVFGRLYALIAAVLFGVATNVKTIHTSKIKEETVHPV

SEQ ID NO: 30 - protein, 729 aa, Bovine
MFEAIRVLQTWAPHMKGLRLALVPGLSCARLGILLFLVLISLPSLYCDLGSPYHSSYEVVIPKSLTVEGREDQVEKLSYVLFMQGQRQLIHLTLKTDYFVDNFPVFSYHDGILGQEMPLISRDCHYEGYIEGVPGSFVSVNTCSGLRGLLIKEGKSYGLEPVHSSKRFEHLLYAMAHEARVSCGVTSKDSQVASTSRRPESGKPHSWQVPSDLWSHTKYVEMFVVVNNQRFQMWGSDVNQTVQRVMDIIALANSFTRGINTEVVLAGMEIWTEGDLTEVPVDLQVALRNFNSWRQEKLFHRVKHDVAHMIVGQHPREDTGQAFLSGACSSDFAAAVESFHHEDVLLFAALMVHELGHNLGIRHDHPACMCKDRPFCLMRENITKESGFSNCSSDFFHRFLWEHKGACLFNKPGHKGRLRRASRCGDGIVEGPEQCDCGSNCERHPCCDTRCQLREHAECSDGLCCDKCRLRYQGFMCRAALGECDLPEYCNGSSGECPRDSYKLDGTMCDRIHYCAGGRCKNPDNQCMDIYGSPARSAPEMCYVSMNTRGDRFGNCGTTSSPRLTYLKCADDNIFCGKLICTNVREIPQLKPNHTLIQVAHKDDWCWSMDAYGTADVPDDGDAHTGTLCAPHKVCMNHLCTDYTSLGYNCETTELCNGKGVCNNFRHCHCEDGYAPPDCKDPGEGGSVDSGPPRISIQLSSGGESETPKRRSYEIQGIGNVVFISLHYF

SEQ ID NO: 31 - protein, 553 aa, Bovine
MRMLRRHHISFRSFAGSSGTPQAVFTFLLLPCCLALDFRAPPLISNTSFLWAWNAPVERCVNRRFQLPPDLRLFSVKGSPQKSATGQFITLFYADRLGYYPHIDEKTGKTVFGGIPQLGNLKSHLEKAKNDIAYYIPNDSVGLAVIDWENWRPTWARNWKPKDVYRDESVELVLQKNPQLSFPEASKIAKVDFETAGKSFMQETLKLGKLLRPNHLWGYYLFPDCYNHNHNQPTYNGNCPDVEKRRNDDLEWLWKESTALFPSVYLNIRLKSTQNAALYVRNRVQEAIRLSKIASVESPLPVFVYARPVFTDGSSTYLSQGDLVNSVGEIVSLGASGIIMWGSLNLSLSMQSCMNLGTYLNTTLNPYIINVTLAAKMCSQVLCHNEGVCTRKHWNSSDYLHLNPMNFAIQTGEGGKYTVPGTVTLEDLQKFSDTFYCSCYANIHCKKRVDIKNVHSVNVCMAEDICIDSPVKLQPSDHSSSQEASTTTFSSISPSTTTATVSPCTPEKHSPECLKVRCSEVIPNVTQKACQSVKLKNISYQSPIQNIKNQTTY

SEQ ID NO: 32 - protein, 524 aa, Bovine
MISPFLLLAIGTCFASSLVPEKEKDPKYWRDQAQQTLKNALRLQTLNTNVAKNVIMFLGDGMGVSTVTAARILKGQLHHSPGEETKLEMDKFPYVALSKTYNTNAQVPDSAGTATAYLCGVKANEGTVGVSAATQRSQCNTTQGNEVTSILRWAKDAGKSVGIVTTTRVNHATPSASYAHSADRDWYSDNEMPPEALSQGCKDIAYQLMHNIKDIEVIMGGGRKYMFPKNRTDVEYELDEKARGTRLDGLNLIDIWKSFKPKHKHSHYVWNRTDLLALDPHSVDYLLGLFEPGDMQYELNRNNATDPSLSEMVEMAIRILNKNPKGFFLLVEGGRIDHGHHEGKAKQALHEAVEMDQAIGQAGAMTSVEDTLTVVTADHSHVFTFGGYTPRGNSIFGLAPMVSDTDKKPFTAILYGNGPGYKVVGGERENVSMVDYAHNNYQAQSAVPLRHETHGGEDVAVFAKGPMAHLLHGVHEQNYIPHVMAYAACIGANRDHCASASSSGSPSPGPLLLLLALLPLGSLF

SEQ ID NO: 33 - protein, 641 aa, Bovine
MAKNMAIGIDLGTTYSCVGVFQHGKVEIIANDQGNRTTPSYVAFTDTERLIGDAAKNQVALNPQNTVFDAKRLIGRKFGDPVVQSDMKHWPFRVINDGDKPKVQVSYKGETKAFYPEEISSMVLTKMKEIAEAYLGHPVTNAVITVPAYFNDSQRQATKDAGVIAGLNVLRIINEPTAAAIAYGLDRTGKGERNVLIFDLGGGTFDVSILTIDDGIFEVKATAGDTHLGGEDFDNRLVNHFVEEFKRKHKKDISQNKRAVRRLRTACERAKRTLSSSTQASLEIDSLFEGIDFYTSITRARFEELCSDLFRSTLEPVEKALRDAKLDKAQIHDLVLVGGSTRIPKVQKLLQDFFNGRDLNKSINPDEAVAYGAAVQAAILMGDKSENVQDLLLLDVAPLSLGLETAGGVMTALIKRNSTIPTKQTQIFTTYSDNQPGVLIQVYEGERAMTRDNNLLGRFELSGIPPAPRGVPQIEVTFDIDANGILNVTATDKSTGKANKITITNDKGRLSKEEIERMVQEAEKYKAEDEVQRERVSAKNALESYAFNMKSAVEDEGLKGKISEADKKKVLDKCQEVISWLDANTLAEKDEFEHKRKELEQVCNPIISRLYQGAGGPGAGGFGAQGPKGGSGSGPTIEEVD

SEQ ID NO: 34 - protein, 126 aa, Bovine
MVLGWLPLLVMVLAPGTTGVKDCVFCELTDSTSCPGTSMRCGDDEDCFTGHGVAPGVGPIINKGCVHATSCGHEEPINYMGVTYSLTTNCCTGHMCNGAPDPTRGRLAGAAASLALGVLLLLQHVL